European Patent Specification EP 4 320 263 B1, published June 19, 2024. Title: Detection of Proximity Assay Products in Situ. Applicant: MOLECULENT AB. Application WO. The sequence listing filed with the application follows.

SEQUENCE LISTING (15 sequences)

SEQ ID NO: 1 - DNA, 36 bp, synthetic construct
  source 1..36: mol_type = other DNA
  modified_base order(4..6,11,16,22,33): mod_base = OTHER; note = deoxyuridine
tttnnngtagncacangacgtngccgaccgtcngtt

SEQ ID NO: 2 - DNA, 36 bp, synthetic construct
  source 1..36: mol_type = other DNA
  modified_base 6: mod_base = OTHER; note = deoxyuridine
tcgacnacaccaaatcgtgcgaagtacggatttttt

SEQ ID NO: 3 - DNA, 20 bp, synthetic construct
  source 1..20: mol_type = other DNA
gtgtagtcgaaacagacggt

SEQ ID NO: 4 - DNA, 60 bp, synthetic construct
  source 1..60: mol_type = other DNA
cggcaacgtcatgtgactacaacccattgttccgcaagcgcgggccgcaaatagctcttt

SEQ ID NO: 5 - DNA, 60 bp, synthetic construct
  source 1..60: mol_type = other DNA
aatgtttcgcgtgcatccggctccaccggatttgcagctttccgtacttcgcacgatttg

SEQ ID NO: 6 - DNA, 36 bp, synthetic construct
  source 1..36: mol_type = other DNA
  modified_base order(4..6,12,14,18,33): mod_base = OTHER; note = deoxyuridine
tttnnncgaaananggancccacgcctgaacanacg

SEQ ID NO: 7 - DNA, 36 bp, synthetic construct
  source 1..36: mol_type = other DNA
  modified_base 6: mod_base = OTHER; note = deoxyuridine
cgtggnagtcccgtggttcggacctaaatctttttt

SEQ ID NO: 8 - DNA, 20 bp, synthetic construct
  source 1..20: mol_type = other DNA
gactaccacgcgtatgttca

SEQ ID NO: 9 - DNA, 60 bp, synthetic construct
  source 1..60: mol_type = other DNA
ggcgtgggatccatatttcgaaatgcccgatcgcaagcgtttggcatgcgacgccaactt

SEQ ID NO: 10 - DNA, 60 bp, synthetic construct
  source 1..60: mol_type = other DNA
tttgaagcaatccgtgggcgggcgcaaacgtttgtcgacagatttaggtccgaaccacgg

SEQ ID NO: 11 - DNA, 36 bp, synthetic construct
  source 1..36: mol_type = other DNA
  modified_base order(4..6,10,32): mod_base = OTHER; note = deoxyuridine
tttnnntatnagcacgccggaaagacagaaanggat

SEQ ID NO: 12 - DNA, 36 bp, synthetic construct
  source 1..36: mol_type = other DNA
  modified_base 3: mod_base = OTHER; note = deoxyuridine
ccncgtagggaatgggcgttcactcttgtatttttt

SEQ ID NO: 13 - DNA, 20 bp, synthetic construct
  source 1..20: mol_type = other DNA
ccctacgaggatccatttct

SEQ ID NO: 14 - DNA, 60 bp, synthetic construct
  source 1..60: mol_type = other DNA
gtctttccggcgtgctaataacacgttgcgcaaaccatcgcaaaccagttggcgcatcgt

SEQ ID NO: 15 - DNA, 60 bp, synthetic construct
  source 1..60: mol_type = other DNA
aatgtttcgcgtgcatccggctccaccggatttgcagctttacaagagtgaacgcccatt